European Patent Application EP 4 306 536 A1, published January 17, 2024. Title: Modified SpoT protein and method for producing L-amino acid using the same. Applicant: CJ CheilJedang Corporation. The sequence listing filed with the application follows.

SEQUENCE LISTING (24 sequences)

SEQ ID NO: 1 - protein, 702 aa, Artificial Sequence
  SpoT_WT
MYLFESLNQLIQTYLPEDQIKRLRQAYLVARDAHEGQTRSSGEPYITHPVAVACILAEMKLDYETLMAALLHDVIEDTPATYQDMEQLFGKSVAELVEGVSKLDKLKFRDKKEAQAENFRKMIMAMVQDIRVILIKLADRTHNMRTLGSLRPDKRRRIARETLEIYSPLAHRLGIHHIKTELEELGFEALYPNRYRVIKEVVKAARGNRKEMIQKILSEIEGRLQEAGIPCRVSGREKHLYSIYCKMVLKEQRFHSIMDIYAFRVIVNDSDTCYRVLGQMHSLYKPRPGRVKDYIAIPKANGYQSLHTSMIGPHGVPVEVQIRTEDMDQMAEMGVAAHWAYKEHGETSTTAQIRAQRWMQSLLELQQSAGSSFEFIESVKSDLFPDEIYVFTPEGRIVELPAGATPVDFAYAVHTDIGHACVGARVDRQPYPLSQPLTSGQTVEIITAPGARPNAAWLNFVVSSKARAKIRQLLKNLKRDDSVSLGRRLLNHALGGSRKLNEIPQENIQRELDRMKLATLDDLLAEIGLGNAMSVVVAKNLQHGDASIPPATQSHGHLPIKGADGVLITFAKCCRPIPGDPIIAHVSPGKGLVIHHESCRNIRGYQKEPEKFMAVEWDKETAQEFITEIKVEMFNHQGALANLTAAINTTTSNIQSLNTEEKDGRVYSAFIRLTARDRVHLANIMRKIRVMPDVIKVTRNRN

SEQ ID NO: 2 - DNA, 2109 bp, Artificial Sequence
  spoT_WT
ttgtatctgtttgaaagcctgaatcaactgattcaaacctacctgccggaagaccaaatcaagcgtctgcggcaggcgtatctcgttgcacgtgatgctcacgaggggcaaacacgttcaagcggtgaaccctatatcacgcacccggtagcggttgcctgcattctggccgagatgaaactcgactatgaaacgctgatggcggcgctgctgcatgacgtgattgaagatactcccgccacctaccaggatatggaacagctttttggtaaaagcgtcgccgagctggtagagggggtgtcgaaacttgataaactcaagttccgcgataagaaagaggcgcaggccgaaaactttcgcaagatgattatggcgatggtgcaggatatccgcgtcatcctcatcaaacttgccgaccgtacccacaacatgcgcacgctgggctcacttcgcccggacaaacgtcgccgcatcgcccgtgaaactctcgaaatttatagcccgctggcgcaccgtttaggtatccaccacattaaaaccgaactcgaagagctgggttttgaggcgctgtatcccaaccgttatcgcgtaatcaaagaagtggtgaaagccgcgcgcggcaaccgtaaagagatgatccagaagattctttctgaaatcgaagggcgtttgcaggaagcgggaataccgtgccgcgtcagtggtcgcgagaagcatctttattcgatttactgcaaaatggtgctcaaagagcagcgttttcactcgatcatggacatctacgctttccgcgtgatcgtcaatgattctgacacctgttatcgcgtgctgggccagatgcacagcctgtacaagccgcgtccgggccgcgtgaaagactatatcgccattccaaaagcgaacggctatcagtctttgcacacctcgatgatcggcccgcacggtgtgccggttgaggtccagatccgtaccgaagatatggaccagatggcggagatgggtgttgccgcgcactgggcttataaagagcacggcgaaaccagtactaccgcacaaatccgcgcccagcgctggatgcaaagcctgctggagctgcaacagagcgccggtagttcgtttgaatttatcgagagcgttaaatccgatctcttcccggatgagatttacgttttcacaccggaagggcgcattgtcgagctgcctgccggtgcaacgcccgtcgacttcgcttatgcagtgcataccgatatcggtcatgcctgcgtgggcgcacgcgttgaccgccagccttacccgctgtcgcagccgcttaccagcggtcaaaccgttgaaatcattaccgctccgggcgctcgcccgaatgccgcttggctgaactttgtcgttagctcgaaagcgcgcgccaaaattcgtcagttgctgaaaaacctcaagcgtgatgattctgtaagcctgggccgtcgtctgctcaaccatgctttgggtggtagccgtaagctgaatgaaatcccgcaggaaaatattcagcgcgagctggatcgcatgaagctggcaacgcttgacgatctgctggcagaaatcggacttggtaacgcaatgagcgtggtggtcgcgaaaaatctgcaacatggggacgcctccattccaccggcaacccaaagccacggacatctgcccattaaaggtgccgatggcgtgctgatcacctttgcgaaatgctgccgccctattcctggcgacccgattatcgcccacgtcagccccggtaaaggtctggtgatccaccatgaatcctgccgtaatatccgtggctaccagaaagagccagagaagtttatggctgtggaatgggataaagagacggcgcaggagttcatcaccgaaatcaaggtggagatgttcaatcatcagggtgcgctggcaaacctgacggcggcaattaacaccacgacttcgaatattcaaagtttgaatacggaagagaaagatggtcgcgtctacagcgcctttattcgtctgaccgctcgtgaccgtgtgcatctggcgaatatcatgcgcaaaatccgcgtgatgccagacgtgattaaagtcacccgaaaccgaaattaa

SEQ ID NO: 3 - DNA, 18 bp, Artificial Sequence
  primer
ccaggaacagcaagagca

SEQ ID NO: 4 - DNA, 18 bp, Artificial Sequence
  primer
acggatattacggcagga

SEQ ID NO: 5 - DNA, 39 bp, Artificial Sequence
  primer
caggaattcgatgtcgcccttgtatctgtttgaaagcct

SEQ ID NO: 6 - DNA, 38 bp, Artificial Sequence
  primer
gctaggtcgactagcgtgatccccatgttgcagatttt

SEQ ID NO: 7 - DNA, 36 bp, Artificial Sequence
  primer
cattgacgatcacgcggaaagagtagatgtccatga

SEQ ID NO: 8 - DNA, 37 bp, Artificial Sequence
  primer
tcgatcatggacatctactctttccgcgtgatcgtca

SEQ ID NO: 9 - DNA, 36 bp, Artificial Sequence
  primer
cattgacgatcacgcggaaagtgtagatgtccatga

SEQ ID NO: 10 - DNA, 37 bp, Artificial Sequence
  primer
tcgatcatggacatctacactttccgcgtgatcgtca

SEQ ID NO: 11 - DNA, 36 bp, Artificial Sequence
  primer
cattgacgatcacgcggaaacagtagatgtccatga

SEQ ID NO: 12 - DNA, 37 bp, Artificial Sequence
  primer
tcgatcatggacatctactgtttccgcgtgatcgtca

SEQ ID NO: 13 - DNA, 36 bp, Artificial Sequence
  primer
cattgacgatcacgcggaaatagtagatgtccatga

SEQ ID NO: 14 - DNA, 37 bp, Artificial Sequence
  primer
tcgatcatggacatctactatttccgcgtgatcgtca

SEQ ID NO: 15 - DNA, 36 bp, Artificial Sequence
  primer
cattgacgatcacgcggaaattgtagatgtccatga

SEQ ID NO: 16 - DNA, 37 bp, Artificial Sequence
  primer
tcgatcatggacatctacaatttccgcgtgatcgtca

SEQ ID NO: 17 - DNA, 36 bp, Artificial Sequence
  primer
cattgacgatcacgcggaattggtagatgtccatga

SEQ ID NO: 18 - DNA, 37 bp, Artificial Sequence
  primer
tcgatcatggacatctaccaattccgcgtgatcgtca

SEQ ID NO: 19 - protein, 702 aa, Artificial Sequence
  SpoT_A262S
MYLFESLNQLIQTYLPEDQIKRLRQAYLVARDAHEGQTRSSGEPYITHPVAVACILAEMKLDYETLMAALLHDVIEDTPATYQDMEQLFGKSVAELVEGVSKLDKLKFRDKKEAQAENFRKMIMAMVQDIRVILIKLADRTHNMRTLGSLRPDKRRRIARETLEIYSPLAHRLGIHHIKTELEELGFEALYPNRYRVIKEVVKAARGNRKEMIQKILSEIEGRLQEAGIPCRVSGREKHLYSIYCKMVLKEQRFHSIMDIYSFRVIVNDSDTCYRVLGQMHSLYKPRPGRVKDYIAIPKANGYQSLHTSMIGPHGVPVEVQIRTEDMDQMAEMGVAAHWAYKEHGETSTTAQIRAQRWMQSLLELQQSAGSSFEFIESVKSDLFPDEIYVFTPEGRIVELPAGATPVDFAYAVHTDIGHACVGARVDRQPYPLSQPLTSGQTVEIITAPGARPNAAWLNFVVSSKARAKIRQLLKNLKRDDSVSLGRRLLNHALGGSRKLNEIPQENIQRELDRMKLATLDDLLAEIGLGNAMSVVVAKNLQHGDASIPPATQSHGHLPIKGADGVLITFAKCCRPIPGDPIIAHVSPGKGLVIHHESCRNIRGYQKEPEKFMAVEWDKETAQEFITEIKVEMFNHQGALANLTAAINTTTSNIQSLNTEEKDGRVYSAFIRLTARDRVHLANIMRKIRVMPDVIKVTRNRN

SEQ ID NO: 20 - protein, 702 aa, Artificial Sequence
  SpoT_A262T
MYLFESLNQLIQTYLPEDQIKRLRQAYLVARDAHEGQTRSSGEPYITHPVAVACILAEMKLDYETLMAALLHDVIEDTPATYQDMEQLFGKSVAELVEGVSKLDKLKFRDKKEAQAENFRKMIMAMVQDIRVILIKLADRTHNMRTLGSLRPDKRRRIARETLEIYSPLAHRLGIHHIKTELEELGFEALYPNRYRVIKEVVKAARGNRKEMIQKILSEIEGRLQEAGIPCRVSGREKHLYSIYCKMVLKEQRFHSIMDIYTFRVIVNDSDTCYRVLGQMHSLYKPRPGRVKDYIAIPKANGYQSLHTSMIGPHGVPVEVQIRTEDMDQMAEMGVAAHWAYKEHGETSTTAQIRAQRWMQSLLELQQSAGSSFEFIESVKSDLFPDEIYVFTPEGRIVELPAGATPVDFAYAVHTDIGHACVGARVDRQPYPLSQPLTSGQTVEIITAPGARPNAAWLNFVVSSKARAKIRQLLKNLKRDDSVSLGRRLLNHALGGSRKLNEIPQENIQRELDRMKLATLDDLLAEIGLGNAMSVVVAKNLQHGDASIPPATQSHGHLPIKGADGVLITFAKCCRPIPGDPIIAHVSPGKGLVIHHESCRNIRGYQKEPEKFMAVEWDKETAQEFITEIKVEMFNHQGALANLTAAINTTTSNIQSLNTEEKDGRVYSAFIRLTARDRVHLANIMRKIRVMPDVIKVTRNRN

SEQ ID NO: 21 - protein, 702 aa, Artificial Sequence
  SpoT_A262C
MYLFESLNQLIQTYLPEDQIKRLRQAYLVARDAHEGQTRSSGEPYITHPVAVACILAEMKLDYETLMAALLHDVIEDTPATYQDMEQLFGKSVAELVEGVSKLDKLKFRDKKEAQAENFRKMIMAMVQDIRVILIKLADRTHNMRTLGSLRPDKRRRIARETLEIYSPLAHRLGIHHIKTELEELGFEALYPNRYRVIKEVVKAARGNRKEMIQKILSEIEGRLQEAGIPCRVSGREKHLYSIYCKMVLKEQRFHSIMDIYCFRVIVNDSDTCYRVLGQMHSLYKPRPGRVKDYIAIPKANGYQSLHTSMIGPHGVPVEVQIRTEDMDQMAEMGVAAHWAYKEHGETSTTAQIRAQRWMQSLLELQQSAGSSFEFIESVKSDLFPDEIYVFTPEGRIVELPAGATPVDFAYAVHTDIGHACVGARVDRQPYPLSQPLTSGQTVEIITAPGARPNAAWLNFVVSSKARAKIRQLLKNLKRDDSVSLGRRLLNHALGGSRKLNEIPQENIQRELDRMKLATLDDLLAEIGLGNAMSVVVAKNLQHGDASIPPATQSHGHLPIKGADGVLITFAKCCRPIPGDPIIAHVSPGKGLVIHHESCRNIRGYQKEPEKFMAVEWDKETAQEFITEIKVEMFNHQGALANLTAAINTTTSNIQSLNTEEKDGRVYSAFIRLTARDRVHLANIMRKIRVMPDVIKVTRNRN

SEQ ID NO: 22 - protein, 702 aa, Artificial Sequence
  SpoT_A262Y
MYLFESLNQLIQTYLPEDQIKRLRQAYLVARDAHEGQTRSSGEPYITHPVAVACILAEMKLDYETLMAALLHDVIEDTPATYQDMEQLFGKSVAELVEGVSKLDKLKFRDKKEAQAENFRKMIMAMVQDIRVILIKLADRTHNMRTLGSLRPDKRRRIARETLEIYSPLAHRLGIHHIKTELEELGFEALYPNRYRVIKEVVKAARGNRKEMIQKILSEIEGRLQEAGIPCRVSGREKHLYSIYCKMVLKEQRFHSIMDIYYFRVIVNDSDTCYRVLGQMHSLYKPRPGRVKDYIAIPKANGYQSLHTSMIGPHGVPVEVQIRTEDMDQMAEMGVAAHWAYKEHGETSTTAQIRAQRWMQSLLELQQSAGSSFEFIESVKSDLFPDEIYVFTPEGRIVELPAGATPVDFAYAVHTDIGHACVGARVDRQPYPLSQPLTSGQTVEIITAPGARPNAAWLNFVVSSKARAKIRQLLKNLKRDDSVSLGRRLLNHALGGSRKLNEIPQENIQRELDRMKLATLDDLLAEIGLGNAMSVVVAKNLQHGDASIPPATQSHGHLPIKGADGVLITFAKCCRPIPGDPIIAHVSPGKGLVIHHESCRNIRGYQKEPEKFMAVEWDKETAQEFITEIKVEMFNHQGALANLTAAINTTTSNIQSLNTEEKDGRVYSAFIRLTARDRVHLANIMRKIRVMPDVIKVTRNRN

SEQ ID NO: 23 - protein, 702 aa, Artificial Sequence
  SpoT_A262N
MYLFESLNQLIQTYLPEDQIKRLRQAYLVARDAHEGQTRSSGEPYITHPVAVACILAEMKLDYETLMAALLHDVIEDTPATYQDMEQLFGKSVAELVEGVSKLDKLKFRDKKEAQAENFRKMIMAMVQDIRVILIKLADRTHNMRTLGSLRPDKRRRIARETLEIYSPLAHRLGIHHIKTELEELGFEALYPNRYRVIKEVVKAARGNRKEMIQKILSEIEGRLQEAGIPCRVSGREKHLYSIYCKMVLKEQRFHSIMDIYNFRVIVNDSDTCYRVLGQMHSLYKPRPGRVKDYIAIPKANGYQSLHTSMIGPHGVPVEVQIRTEDMDQMAEMGVAAHWAYKEHGETSTTAQIRAQRWMQSLLELQQSAGSSFEFIESVKSDLFPDEIYVFTPEGRIVELPAGATPVDFAYAVHTDIGHACVGARVDRQPYPLSQPLTSGQTVEIITAPGARPNAAWLNFVVSSKARAKIRQLLKNLKRDDSVSLGRRLLNHALGGSRKLNEIPQENIQRELDRMKLATLDDLLAEIGLGNAMSVVVAKNLQHGDASIPPATQSHGHLPIKGADGVLITFAKCCRPIPGDPIIAHVSPGKGLVIHHESCRNIRGYQKEPEKFMAVEWDKETAQEFITEIKVEMFNHQGALANLTAAINTTTSNIQSLNTEEKDGRVYSAFIRLTARDRVHLANIMRKIRVMPDVIKVTRNRN

SEQ ID NO: 24 - protein, 702 aa, Artificial Sequence
  SpoT_A262Q
MYLFESLNQLIQTYLPEDQIKRLRQAYLVARDAHEGQTRSSGEPYITHPVAVACILAEMKLDYETLMAALLHDVIEDTPATYQDMEQLFGKSVAELVEGVSKLDKLKFRDKKEAQAENFRKMIMAMVQDIRVILIKLADRTHNMRTLGSLRPDKRRRIARETLEIYSPLAHRLGIHHIKTELEELGFEALYPNRYRVIKEVVKAARGNRKEMIQKILSEIEGRLQEAGIPCRVSGREKHLYSIYCKMVLKEQRFHSIMDIYQFRVIVNDSDTCYRVLGQMHSLYKPRPGRVKDYIAIPKANGYQSLHTSMIGPHGVPVEVQIRTEDMDQMAEMGVAAHWAYKEHGETSTTAQIRAQRWMQSLLELQQSAGSSFEFIESVKSDLFPDEIYVFTPEGRIVELPAGATPVDFAYAVHTDIGHACVGARVDRQPYPLSQPLTSGQTVEIITAPGARPNAAWLNFVVSSKARAKIRQLLKNLKRDDSVSLGRRLLNHALGGSRKLNEIPQENIQRELDRMKLATLDDLLAEIGLGNAMSVVVAKNLQHGDASIPPATQSHGHLPIKGADGVLITFAKCCRPIPGDPIIAHVSPGKGLVIHHESCRNIRGYQKEPEKFMAVEWDKETAQEFITEIKVEMFNHQGALANLTAAINTTTSNIQSLNTEEKDGRVYSAFIRLTARDRVHLANIMRKIRVMPDVIKVTRNRN